European Patent Specification EP 3 988 665 B1, published August 30, 2023. Title: METHOD AND USE FOR CONSTRUCTION OF SEQUENCING LIBRARY BASED ON DNA SAMPLES. Applicant: MGI TECH CO., LTD. The sequence listing filed with the application follows.

SEQUENCE LISTING (26 sequences)

SEQ ID NO: 1 - DNA, 58 bp, Artificial Sequence
  Adapter 1
  misc_feature (1)..(1): phosphorylation
  misc_feature (32)..(41): n is a, c, g, or t
agtcggaggccaagcggtcttaggaagacaannnnnnnnnncaactccttggctcaca

SEQ ID NO: 2 - DNA, 37 bp, Artificial Sequence
  Adapter 2
agccaaggtcagtaacgacatggctacgatccgactt

SEQ ID NO: 3 - DNA, 17 bp, Artificial Sequence
  Universal primer 1
  misc_feature (1)..(1): phosphorylation
gaacgacatggctacga

SEQ ID NO: 4 - DNA, 17 bp, Artificial Sequence
  Universal primer 2
tgtgagccaaggagttg

SEQ ID NO: 5 - DNA, 25 bp, Artificial Sequence
  Universal primer 3
  misc_feature (1)..(1): phosphorylation
gaacgacatggctacgatccgactt

SEQ ID NO: 6 - DNA, 59 bp, Artificial Sequence
  Universal primer 4
  misc_feature (18)..(27): n is a, c, g, or t
tgtgagccaaggagttgnnnnnnnnnnttgtcttcctaagaccgcttggcctccgactt

SEQ ID NO: 7 - DNA, 49 bp, Artificial Sequence
  Specific primer
acatggctacgatccgacttgatgtgtttgggatattgtttattttatg

SEQ ID NO: 8 - DNA, 40 bp, Artificial Sequence
  Specific primer
acatggctacgatccgactttgtgtgttgtggtgaggagg

SEQ ID NO: 9 - DNA, 40 bp, Artificial Sequence
  Specific primer
acatggctacgatccgacttaggagggaaggtttgaggtt

SEQ ID NO: 10 - DNA, 44 bp, Artificial Sequence
  Specific primer
acatggctacgatccgacttggttagttggaaggagtggaaatt

SEQ ID NO: 11 - DNA, 39 bp, Artificial Sequence
  Specific primer
acatggctacgatccgacttacgtgaaaggggagaggta

SEQ ID NO: 12 - DNA, 41 bp, Artificial Sequence
  Specific primer
acatggctacgatccgacttggagtttttttgtggggtgag

SEQ ID NO: 13 - DNA, 42 bp, Artificial Sequence
  Specific primer
acatggctacgatccgacttggtggggtaaaggtgattttag

SEQ ID NO: 14 - DNA, 47 bp, Artificial Sequence
  Specific primer
acatggctacgatccgacttagtttttttagatgttgtgaattgggg

SEQ ID NO: 15 - DNA, 43 bp, Artificial Sequence
  Specific primer
acatggctacgatccgactttgtggtgtagttagaagtggttt

SEQ ID NO: 16 - DNA, 43 bp, Artificial Sequence
  Specific primer
acatggctacgatccgacttggagggttggtaaagtttagaag

SEQ ID NO: 17 - DNA, 37 bp, Artificial Sequence
  Specific primer
cgcttggcctccgacttcaaatggcagcagaggaatc

SEQ ID NO: 18 - DNA, 36 bp, Artificial Sequence
  Specific primer
cgcttggcctccgacttgaatggatggcttggcctg

SEQ ID NO: 19 - DNA, 40 bp, Artificial Sequence
  Specific primer
cgcttggcctccgacttgtcttctagtggaagaagtgaac

SEQ ID NO: 20 - DNA, 38 bp, Artificial Sequence
  Specific primer
cgcttggcctccgacttgtctgacttaagactggtggc

SEQ ID NO: 21 - DNA, 41 bp, Artificial Sequence
  Specific primer
cgcttggcctccgactttcagtgtacctaacacaatatagg

SEQ ID NO: 22 - DNA, 40 bp, Artificial Sequence
  Specific primer
cgcttggcctccgacttagacataggtatgacaagttgca

SEQ ID NO: 23 - DNA, 35 bp, Artificial Sequence
  Specific primer
cgcttggcctccgacttcctgatcccagggtgctg

SEQ ID NO: 24 - DNA, 37 bp, Artificial Sequence
  Specific primer
cgcttggcctccgacttagacccagtgacaaaatgcc

SEQ ID NO: 25 - DNA, 42 bp, Artificial Sequence
  specific primer
cgcttggcctccgacttcttacttaaccattgtgtccttccc

SEQ ID NO: 26 - DNA, 40 bp, Artificial Sequence
  Specific primer
cgcttggcctccgacttctccaaagaatgattcctcattc